European Patent Application EP 4 292 584 A1, published December 20, 2023. Title: COMPOSITION FOR MICRONEEDLE ADMINSTRATION AND IT'S APPLICATIONS. Applicant: Zcapsule Pharmaceuticals Co., Ltd. The sequence listing filed with the application follows.

SEQUENCE LISTING (1 sequence)

SEQ ID NO: 1 - RNA, 2163 nt, synthetic construct
  source 1..2163: mol_type = other RNA
tctcaacacaacatatacaaaacaaacgaatctcaagcaatcaagcattctacttctattgcagcaatttaaatcatttcttttaaagcaaaagcaattttctgaaaattttcaccatttacgaacgatagcatgggctggtcctgcatcatcttgttcttggtggctactgccactggagtacacagcgagattgtccttacacagtcaccaggcaccctttccttgtctcctggggaacgagccaccctcagttgtcggtcaagcaagaatctgctgcattccaatgggatcacatacctgtattggtaccagcagaagcctggacaggcacccagactgctcatctaccagatgtccaatctggcctcaggcattcctgacaggttttccggcagcgggtctggcaccgatttcaccctgaccatatccaggctcgaaccagaggattttgccgtgtattactgcgcacagaatctggagattccccgcacttttggccaagggactaaactggagatcaagcggggaggaggcggctctggaggtggcggcagtggtggaggcgggtctggcggtggcggatctggaggtggtgggagccaggtccagcttgttcagtcaggcgcagaggtgaagaaacccggagctagcgtgaaagtctcctgcaaagcgtcagggtacaccttcaccaactatgggatgaactgggtacgtcaagccccagggcaaagactcgaatggatgggttggatcaacacgtacacaggggaaccgacttatggcgaggacttcaaggggagagtgaccataacactggacacatccgctagcacagcgtatatggagctgagcagtctgaggagcgaagatacggctgtttactattgtgcccgctttggtaactacgtggactattggggtcagggaactctggtgacggtttctagcagtggcggcggaggatcccaggtgcagctgcagcagtctggcgctgagctggctagacctggcgcctccgtgaagatgtcctgcaagacctccggctacaccttcacccggtacaccatgcactgggtcaagcagaggcctggacagggcctggaatggatcggctacatcaacccctcccggggctacaccaactacaaccagaagttcaaggacaaggccaccctgacaaccgacaagtcctcctccaccgcctacatgcagctgtcctccctgacctccgaggactccgccgtgtactactgcgcccggtactacgacgaccactactccctggactactggggccagggcaccacactgacagtgtctagcggaggcggaggatctggtggtggcggatctggcggcggtggaagtggcggaggtggtagccagatcgtgctgacccagtctcccgccatcatgtctgctagccctggcgagaaagtgacaatgacctgccgggcctcctcctccgtgtcctacatgaactggtatcagcagaagtccggcacctcccccaagcggtggatctacgacacctccaaggtggcctctggcgtgccctacagattctccggctctggctctggcacctcctacagcctgaccatctccagcatggaagccgaggatgccgccacctactactgccagcagtggtcctccaaccccctgacctttggcgctggcaccaagctggaactgaagggcggctctcaccaccaccatcaccactgatgagctgcagaattcgtcgacggatccgatctggtactgcatgcacgcaatgctagctgcccctttcccgtcctgggtaccccgagtctcccccgacctcgggtcccaggtatgctcccacctccacctgccccactcaccacctctgctagttccagacacctcccaagcacgcagcaatgcagctcaaaacgcttagcctagccacacccccacgggaaacagcagtgattaacctttagcaataaacgaaagtttaactaagctatactaaccccagggttggtcaatttcgtgccagccacaccctcgagctagcaaaaaaaaaaaaaaaaaaaaaaaaaaaaaagcatatgactaaaaaaaaaaaaaaaaaaaaaaaaaaaaaaaaaaaaaaaaaaaaaaaaaaaaaaaaaaaaaaaaaaaaaa